European Patent Application EP 4 394 036 A1, published July 3, 2024. Title: 酶固定化载体及其制备方法、固定化酶及其制备方法. Applicant: 辽宁凯莱英医药化学有限公司. The sequence listing filed with the application follows.

SEQUENCE LISTING (11 sequences)

SEQ ID NO: 1 - protein, 459 aa, Chromobacterium violaceum DSM30191
MQKQRTTSQWRELDAAHHLHPFTDTASLNQAGARVMTRGEGVYLWDSEGNKIIDGMAGLWCVNVGYGRKDFAEAARRQMEELPFYNTFFKTTHPAVVELSSLLAEVTPAGFDRVFYTNSGSESVDTMIRMVRRYWDVQGKPEKKTLIGRWNGYHGSTIGGASLGGMKYMHEQGDLPIPGMAHIEQPWWYKHGKDMTPDEFGVVAARWLEEKILEIGADKVAAFVGEPIQGAGGVIVPPATYWPEIERICRKYDVLLVADEVICGFGRTGEWFGHQHFGFQPDLFTAAKGLSSGYLPIGAVFVGKRVAEGLIAGGDFNHGFTYSGHPVCAAVAHANVAALRDEGIVQRVKDDIGPYMQKRWRETFSRFEHVDDVRGVGMVQAFTLVKNKAKRELFPDFGEIGTLCRDIFFRNNLIMRACGDHIVSAPPLVMTRAEVDEMLAVAERCLEEFEQTLKARGLA

SEQ ID NO: 2 - protein, 459 aa, Chromobacterium violaceum DSM30191; identical to SEQ ID NO: 1

SEQ ID NO: 3 - protein, 476 aa, Arthrobacter citreus
MGLTVQKINWEQVKEWDRKYLMRTFSTQNEYQPVPIESTEGDYLITPGGTRLLDFFNQLCCVNLGQKNQKVNAAIKEALDRYGFVWDTYATDYKAKAAKIIIEDILGDEDWPGKVRFVSTGSEAVETALNIARLYTNRPLVVTREHDYHGWTGGAATVTRLRSFRSGLVGENSESFSAQIPGSSCSSAVLMAPSSNTFQDSNGNYLKDENGELLSVKYTRRMIENYGPEQVAAVITEVSQGVGSTMPPYEYVPQIRKMTKELGVLWISDEVLTGFGRTGKWFGYQHYGVQPDIITMGKGLSSSSLPAGAVVVSKEIAAFMDKHRWESVSTYAGHPVAMAAVCANLEVMMEENLVEQAKNSGEYIRSKLELLQEKHKSIGNFDGYGLLWIVDIVNAKTKTPYVKLDRNFRHGMNPNQIPTQIIMEKALEKGVLIGGAMPNTMRIGASLNVSRGDIDKAMDALDYALDYLESGEWQQS

SEQ ID NO: 4 - protein, 341 aa, Actinobacteria
MTISKDIDYSTSNLVSVAPGAIREPTPAGSVIQYSDYELDESSPFAGGAAWIEGEYVPAAEARISLFDTGFGHSDLTYTVAHVWHGNIFRIKDHIDRVFDGAQKLRLQSPITKAEVEDITKRCVSLSQLRESFVNITITRGYGARKGEKDLSKLTSQIYIYAIPYLWAFPPEEQIFGTSAIVPRHVRRAGRNTVDPTVKNYQWGDLTAASFEAKDRGARTAILLDADNCVAEGPGFNVVMVKDGKLSSPSRNALPGITRLTVMEMADEMGIEFTLRDITSRELYEADELIAVTTAGGITPITSLDGEPLGDGTPGPVTVAIRDRFWAMMDEPSSLVEAIEY

SEQ ID NO: 5 - protein, 338 aa, Sciscionella sp. SE31
MTTTEFANSNLVAVEPGAIREPTPPGSVIQYSEYELDRSQPLAGGVAWIEGEYVPADEARISIFDTGFGHSDLTYTVAHVWHGNIFRLEDHLDRLLHGAARLKLETGMSREELAGIAKRCVSLSQLREAYVNITITRGYGKKRGEKDLTKLTHQVYVYAIPYLWAFPPEEQIFGTSVIVPRHVRRAGRNTIDPTIKNYQWGDLTAASFEAKDRGARSAVLLDADNCVAEGPGFNVVLVKDGALVSPSRNALPGITRKTVYEIAAAKGIETMLRDVTSSELYEADELMAVTTAGGVTPITSLDGEQVGNGEPGPITVAIRDRFWALMDEPSSLIEAIDY

SEQ ID NO: 6 - protein, 253 aa, Acetobacter sp. CCTCC M209061
MARVAGKVAIVSGAANGIGKATAQLLAKEGAKVVIGDLKEEDGQKAVAEIKAAGGEAAFVKLNVTDEAAWKAAIGQTLKLYGRLDIAVNNAGINYSGSVESTSLEDWRRVQSINLDGVFLGTQVAIEAMKKSGGGSIVNLSSISGLIGDPMLAAYVASKGGVRLFTKSAALHCAKSGYKIRVNSVHPGYIWTPMVAGLTKEDAAARQKLVDLHPIGHLGEPNDIAYGILYLASDESKFVTGSELVIDGGYTAQ

SEQ ID NO: 7 - protein, 603 aa, Rhodococcus ruber-SD1
MTTSIDREALRRKYAEERDKRIRPDGNDQYIRLDHVDGWSHDPYMPITPREPKLDHVTFAFIGGGFSGLVTAARLRESGVESVRIIDKAGDFGGVWYWNRYPGAMCDTAAMVYMPLLEETGYMPTEKYAHGPEILEHCQRIGKHYDLYDDALFHTEVTDLVWQEHDQRWRISTNRGDHFTAQFVGMGTGPLHVAQLPGIPGIESFRGKSFHTSRWDYDYTGGDALGAPMDKLADKRVAVIGTGATAVQCVPELAKYCRELYVVQRTPSAVDERGNHPIDEKWFAQIATPGWQKRWLDSFTAIWDGVLTDPSELAIEHEDLVQDGWTALGQRMRAAVGSVPIEQYSPENVQRALEEADDEQMERIRARVDEIVTDPATAAQLKAWFRQMCKRPCFHDDYLPAFNRPNTHLVDTGGKGVERITENGVVVAGVEYEVDCIVYASGFEFLGTGYTDRAGFDPTGRDGVKLSEHWAQGTRTLHGMHTYGFPNLFVLQLMQGAALGSNIPHNFVEAARVVAAIVDHVLSTGTSSVETTKEAEQAWVQLLLDHGRPLGNPECTPGYYNNEGKPAELKDRLNVGYPAGSAAFFRMMDHWLAAGSFDGLTFR

SEQ ID NO: 8 - protein, 541 aa, Rhodococcus sp. Phi1
MTAQISPTVVDAVVIGAGFGGIYAVHKLHNEQGLTVVGFDKADGPGGTWYWNRYPGALSDTESHLYRFSFDRDLLQDGTWKTTYITQPEILEYLESVVDRFDLRRHFRFGTEVTSAIYLEDENLWEVSTDKGEVYRAKYVVNAVGLLSAINFPDLPGLDTFEGETIHTAAWPEGKNLAGKRVGVIGTGSTGQQVITALAPEVEHLTVFVRTPQYSVPVGNRPVTKEQIDAIKADYDGIWDSVKKSAVAFGFEESTLPAMSVSEEERNRIFQEAWDHGGGFRFMFGTFGDIATDEAANEAAASFIRSKIAEIIEDPETARKLMPTGLYAKRPLCDNGYYEVYNRPNVEAVAIKENPIREVTAKGVVTEDGVLHELDVLVFATGFDAVDGNYRRIEIRGRNGLHINDHWDGQPTSYLGVTTANFPNWFMVLGPNGPFTNLPPSIETQVEWISDTVAYAERNEIRAIEPTPEAEEEWTQTCTDIANATLFTRGDSWIFGANVPGKKPSVLFYLGGLGNYRNVLAGVVADSYRGFELKSAVPVTA

SEQ ID NO: 9 - protein, 537 aa, Brachymonas petroleovorans
MSSSPSSAIHFDAIVVGAGFGGMYMLHKLRDQLGLKVKVFDTAGGIGGTWYWNRYPGALSDTHSHVYQYSFDEAMLQEWTWKNKYLTQPEILAYLEYVADRLDLRPDIQLNTTVTSMHFNEVHNIWEVRTDRGGYYTARFIVTALGLLSAINWPNIPGRESFQGEMYHTAAWPKDVELRGKRVGVIGTGSTGVQLITAIAPEVKHLTVFQRTPQYSVPTGNRPVSAQEIAEVKRNFSKVWQQVRESAVAFGFEESTVPAMSVSEAERQRVFQEAWNQGNGFYYMFGTFCDIATDPQANEAAATFIRNKIAEIVKDPETARKLTPTDVYARRPLCDSGYYRTYNRSNVSLVDVKATPISAMTPRGIRTADGVEHELDMLILATGYDAVDGNYRRIDLRGRGGQTINEHWNDTPTSYVGVSTANFPNMFMILGPNGPFTNLPPSIEAQVEWITDLVAHMRQHGLATAEPTRDAEDAWGRTCAEIAEQTLFGQVESWIFGANSPGKKHTLMFYLAGLGNYRKQLADVANAQYQGFAFQPL

SEQ ID NO: 10 - protein, 366 aa, Thermoactinomyces intermedius ATCC33205
MRDVFEMMDRYGHEQVIFCRHPQTGLKAIIALHNTTAGPALGGCRMIPYASTDEALEDVLRLSKGMTYKCSLADVDFGGGKMVIIGDPKKDKSPELFRVIGRFVGGLNGRFYTGTDMGTNPEDFVHAARESKSFAGLPKSYGGKGDTSIPTALGVFHGMRATARFLWGTDQLKGRVVAIQGVGKVGERLLQLLVEVGAYCKIADIDSVRCEQLKEKYGDKVQLVDVNRIHKESCDIFSPCAKGGVVNDDTIDEFRCLAIVGSANNQLVEDRHGALLQKRSICYAPDYLVNAGGLIQVADELEGFHEERVLAKTEAIYDMVLDIFHRAKNENITTCEAADRIVMERLKKLTDIRRILLEDPRNSARR

SEQ ID NO: 11 - protein, 301 aa, Thermosyntropha lipolytica
MGEKIRVAIVGYGNIGRYALDAIKAAPDMELAGVVRRSSSLGDKPAELADVPVVGSIKELTGVKVALLCTPTRSVPEYAREILALGINTVDSYDIHGQLADLRLELDKVAKEHNAVAVISAGWDPGTDSMVRCMFEFMAPKGITYTNFGPGMSMGHSVAVKAVKGVKNALSMTIPLGTGVHRRMVYVELEPGADFAQVEKAVKTDPYFVKDETHVIQVEDVDALIDMGHGVLMERKGVSGGTHNQLLSFSMRINNPALTAQIMVASARASVKQKPGAYTMIQIPIIDYMYGDPDEIIRQLV